European Patent Application EP 4 488 351 A1, published January 8, 2025. Title: CLEANING COMPOSITIONS CONTAINING PORPHYRIN BINDING PROTEINS. Applicant: Procter & Gamble. Application EP. The sequence listing filed with the application follows.

SEQUENCE LISTING (23 sequences)

SEQ ID NO: 1 - protein, 206 aa, Flavobacterium collinsii
MTKIITVITLFICSLLSAQTQFEQGMNKAFGLWKEGKNAEASAMFERIAAAEKTSWLPNYYVGLVNTLSVFTEKDKTKIELLLVKAQDAVDAEMLKDQSNSELYVLQALIYTGYVVADPMTNGMKYSGKVMEAYAKAKALDPNNPRAVFGEADYQLGGAKWTGVDTKPLCAQVNKAIELFGTFKPETPFSPKWGLERALEVQKTCK

SEQ ID NO: 2 - protein, 206 aa, Flavobacterium crocinum
MTKIITVITLFICSLLSAQTQFEQGMNKAFGLWKEGKNAEASAMFERIAAAEKTSWLPNYYVGLVNTLAVFSEKDKTKIELLLVKAQDAVDAEMLKDQSNSELYVLQALIYTGYVVADPMTNGMKYSGKVMEAYAKAKALDPNNPRAVFGEADYQLGGAKWTGVDTKPLCAQVNKAIELFGTFKPETPFSPKWGLERALEVQKTCK

SEQ ID NO: 3 - protein, 206 aa, Flavobacterium cutihirudinis
MTKIITVITLFICSLLSGQTQFEQGMTKAFGLWKEGKNTEASAMFERIAAAEKNSYLPNYYIALINATAVFTEKDKTKIDLLLTKAQDALDIEMIKDQSNSELYVMQALIYTGYVVADPMTNGMKYSGKVMEAYAKAKALDPNNPRAVFGEADYQLGGAKWTGVDTKPLCAQVDKSIELFGTFKPATPFSPKWGLERALEIQKTCK

SEQ ID NO: 4 - protein, 207 aa, Flavobacterium daemonense
MKKIVTLIALFVVVISSAQTQFEQGMGKAFGLWKEGKNAEASAMFERIAAAEKTSYLPNYYVALINTTSAFSEKDKTKIDLLLTKAQDALDVEMIKDQNNAELYAMQALIYTAWVVADPMTNGMKYSAKVMEAYAKGKAIDPNNPRIVFGEADYQIGGAKWSGVDTKPLCAQVDRAVELFTTFKPATPFSPKWGIERALETQKNCKK

SEQ ID NO: 5 - protein, 206 aa, Flavobacterium sp. F-29
MTKMITSIALFVCSLLSAQGQFEQGMGKAFGLWKEGKTTEASDLFERIAAAEKSSWLPNYYVALVNTTTAFGTSDKEKISLLLSKAQNALDVELLKDTNNAELYVMQAMINTAWIVADPMVNGMKLSGKVMELYTKAEALAPDNPRVVFSKADFQINGAKWTGADTKPLCAQLEKAIGLFATFKPENAFSPKWGLDRATAALKNCK

SEQ ID NO: 6 - protein, 208 aa, Flavobacterium gossypii
MTKFILTIAFFITTLAGAQTQYEQGMQKAFALWGEGKTTEASALFERIASAEKNNWLPNYYVALVNTTTAFQTQDKNQIVALLGKAQEALNTELDKNPENPELLVMQAMINTAWIVADPMTNGMKLSAKTIEIYDKALKIAPENPRALFSKAEFEIGGARYFGNDTKPMCAQIDKAIELFAKFKPETPFHPNWGLDRALEAQKECNKK

SEQ ID NO: 7 - protein, 208 aa, Flavobacterium sp.
MTKIITFIALFIASIVLGQTNYEKGMQDALSLWKNKKPSEATAILERIASVEEGNWLPNYYIALINTTQSFRYMDDKSKVKILLETAQKAQDKINIIAPDNPEVLVMQAMIHTAWIVYDPMANGQKLSGDIMYIYNKAYKLAPENPRVVFSKADFEMGMASYFGQDTKPMCAEIEKSLELFANFIPKTPFHPTWGLDRANETSEKCKK

SEQ ID NO: 8 - protein, 218 aa, Porphyromonas gingivalis
MKTFKRIALLLVAGFAGLCATSAQGTAYAEVMNRKVAALDSVPPTEYATLAADFSRIAAVEGSDWMAAYYTAYCRIIPAFGNPSEADRLCEEAESMLSKAESLGGDLSEIACLRSMAASARLLVNPQERWQTYGAESSRQLAVALEANPANPRAYFLQAQSLLYTPAQFGGGKDKALPFAEKSVSCYAAATVSPAYAPHWGEQQARQLLMLCKAETQE

SEQ ID NO: 9 - protein, 218 aa, Porphyromonas gulae
MKTFKRIALLLVAGFAGLCATYAQGTAYAEVMNRKVAALDSVPPTEYATLAADFSRIAAVEGSDWMAAYYAAYCRIIPAFGNPSEADRLCAEAESMLSKAESLGGDLSEIACLRSMAASARLLVNPQERWQTYGVESSRQLAVALEANPANPRAYFLQAQSLLYTPAQFGGGKDKALPFAEKSVSCYAAATVSPAYAPHWGEQQARQLLMLCKAESQE

SEQ ID NO: 10 - protein, 209 aa, Sphingobacteriales bacterium
MKKLIFSLALLVSIAASAQSDKYTQMMQKNIALLDSAKSIDDLQSLASTFDRIGDAEKTKWLPYYYAALAQTWVGWNPTVQDKDANSAKINAYLAKAEALEKNSELYAVENMSATQQMLVDPQTRWATYGKTAGEALQKGLQADPNNPRLYYLQGMSLFGTPTQFGGGKDKAKPLFEKSVSLYKTAHPEPLAPTWGQQQAEAMLEQCGK

SEQ ID NO: 11 - protein, 928 aa, Haemophilus influenzae
MYKLNVISLIILTTCSGAAYASTPDFPQHHKTVFGTVTIEKTTADKMTIKQGSDKAQIDWKSFDIGQKKEVKFEQPNEHAVAYNRVIGGNASQIQGKLTANGKVYLANPNGVIITQGAEINVAGLLATTKDLERISENSNSYQFTRRTKDRQVLKEGLVLKDGQVVKEGQVINEGNITAQDFVVLNGDEVINKGNINVEKNSTINGKVYLSSGYNFTFTLPDSGISVALEDNTVQGIVKNEGSIKAGEITLSAKGRKQALDSLVMNNGVLEATKVSNKNGKVVLSADNVELNNESNIKGEIVTFGADVTSNKELKDNIKITSKTGSKVTSPKINFTGKSVNINGNFGREDSTTHYKDEFKKLNTEVNIDVPDNENIRIADIEDNTGTGTTGTGTSSFIQTGALSSLLANNGKVNLKGNNVNISGRIHIDSFRGSDSLLKLTNKGHIDINNADIHSKGRLFFITSLQNEEDFKSNITITDSKINLGNGAMGLGRSVDEKDYDNRWQKTEGSQRKKFDVKMSNVEFNQVDDVILAGGFEKVNLDKIVATGQTNFYIDGGVSRNGRKYEYGVLDLDKRTQLSELNQGRRRWGYYYDLELDMNRAYLYRFDLFATKNTGRSTIKDTEINISNSNINLKNGFVHLLAEKIKLDNSKIDITFDKDNSQDTLAQTNRLGMNGKVSMINSHIKIVGDEKEGISPTGTYATMFLIGELIGEKSSIFVKSHQGYTFKTDGNTKIAGKYSKEDLKITAINTGGRAAEEVLINGALGSADNDANIANMAFTIGDSANTKTTIENADITALAPNGGTAYLSSKDVEIEVKPNSNFTFFELPREKNLNQTKINGASTKLSERGFARLYDKINGVRASNLSAEQLNVTDASEKIINTKLVSSLDVEKLVSVAVCDAGNGCEEQQFGDKGNNTKVSVGELEAEQ

SEQ ID NO: 12 - protein, 316 aa, Staphylococcus aureus
MTKHYLNSKYQSEQRSSAMKKITMGTASIILGSLVYIGADSQQVNAATEATNATNNQSTQVSQATSQPINFQVQKDGSSEKSHMDDYMQHPGKVIKQNNKYYFQTVLNNASFWKEYKFYNANNQELATTVVNDNKKADTRTINVAVEPGYKSLTTKVHIVVPQINYNHRYTTHLEFEKAIPTLADAAKPNNVKPVQPKPAQPKTPTEQTKPVQPKVEKVKPTVTTTSKVEDNHSTKVVSTDTTKDQSQTQSARTVKTTQTAQEQNKVQTPVKDVATAKSESNSQAVSDNKSQQTNKVTKQNETPKQASKAKELPKT

SEQ ID NO: 13 - protein, 216 aa, Porphyromonas gingivalis
MKKIIFSALCALPLIVSLTSCGKKKDEPNQPSTPEAVTKTVTIDASKYETWQYFSFSKGEVVNVTDYKNDLNWDMALHRYDVRLNCGESGKGKGGAVFSGKTEMDQATTVPTDGYTVDVLGRITVKYEMGPDGHQMEYEEQGFSEVITGKKNAQGFASGGWLEFSHGPAGPTYKLSKRVFFVRGADGNIAKVQFTDYQDAELKKGVITFAYTYPVK

SEQ ID NO: 14 - protein, 225 aa, Prevotella intermedia
MKTKIFAVACLATLLFTSCSKDNNDDPNPKPETTQVKHFETLMPGYDSWIYIDLETGKFEQQAELGKREFRKYKSMMDPNYEVVGTEPAKGTDADLPKKWDIAFHITDARTNNGEVLMTGETDLNKINALPAGNYVADAPADIVVDMSRMQSEGVLGMVKTMLNGEMGKWVKSNGMGKPKTVMGNVFAVKFKNGNAALIKFKDNLDKTGKKKAVSFDYKFIKKAK

SEQ ID NO: 15 - protein, 246 aa, Prevotella intermedia
MKFKSFMALSCLTVLLFSSCSNDDPTPKPKPEQPKDVPTKTLSFITQEKAFQGYDKWVYVNLETGETVMKDDVSEQEWRTYSDAGKKKDLFGKYDVTKTVEGKPSNAPDKWHLAFHVFDVRTNGAEACMTDTTDIETIKTLPTNVKWVSDIKAYLIYDMTGMMKNPVVMGYMKSYVNMGLYYWMHKVKGTMGEYALTMSKSDPKKAPVFLVKFKDGSYAVIQFTGLKDATGKKKEVSFKYKFVKKN

SEQ ID NO: 16 - protein, 336 aa, Streptococcus gordonii
MVVKVGINGFGRIGRLAFRRIQNVEGVEVTRINDLTDPVMLAHLLKYDTTQGRFDGTVEVKEGGFEVNGKFVKVSAERDPENIDWANDGVEIVLEATGFFATKAAAEKHLHAGGAKKVVITAPGGSDVKTVVFNTNHDILDGTETVISGASCTTNCLAPMAKALQDNFGVVEGLMTTIHAYTGDQMILDGPHRKGDLRRARAGAANIVPNSTGAAKAIGLVIPELNGKLDGAAQRVPTPTGSVTELVVVLEKNVTVDEVNAAMKAVANESYGYTEDPIVSSDVVGMSYGSLFDATQTKVLDVDGKQLVKVVSWYDNEMSYTAQLVRTLEYFAKIAK

SEQ ID NO: 17 - protein, 272 aa, Haemophilus haemolyticus
MSVINKTILAVVVCGVVSVAQAQVVGNVSTDTNQTRYIKIKAGEKDGKAGVEIYDSSIPNDPAVLSKTANNKGQSFEKMAERADKWISHLTGVAKKDKNGVIVAKMNKMPNLTLIMPDHRGLGRLSFKQVGNQDTYFGEWENVDAATSAAKNVSVYYAGSDPTKTLPSGKATYTVEGINKYGNFNSRLMKGTFDVDFERASISGYLSKPNLSLSIESKIDKTNATFEGIAKAEGVIGKSEGRFYGAKAEGLAGMATFASKPEYNTAFGGTKN

SEQ ID NO: 18 - protein, 569 aa, Listeria marthii
MKKLWKKGLVAFLALTLIFQLIPGFANAADSRLKDGGEYQVQVNFYKDNTGKTTKESSEADKYIDHTATIKVENGQPYMYLTITNSSWWQTMAVSKDGTRPEKPAQAEVYQAGYQDVQTVSTDAAKDTRVEKFKLSSLDDVIFSYMHIKVDAISYDHWYQVDLTIDPSTFKVISEPAVTTPVTLSDGIYTIPFVAKKANDDSNSSMQNYFNNPAWLKVKNGKKMVAMTVNDNKTVTALKTNLAGALQDVKVVSEDKDANTRIVEFEVEDLNQPLAAHVNYEAPFNGSVYKGQADFRYVFDTTKAVVASSYPGSDETPPVVDPGETNPPVTTPDPGTTNPPVTTPPTTPSKPVVVDPKNLLNNHTYSIDFDVFKDGTTETSMMESYVMKPAVIKVENNQPYVYLTLTNSSWIKTFQYKQNGVWKDMEVVSGDINKNTRTVKYPVKDGTANTDVKTHVLIEDMPGFAYDHEYTVQVKLNAATIKDITGKDVTLKEPVKNDLLNMGNVANNNNAGPKLAKPDFDDTNSVQKTANKAEKNAKTNDSSSMAWYVTLFGASFLYLAYRLKRKRLS

SEQ ID NO: 19 - protein, 261 aa, Acinetobacter baumannii
MSQLFLGLVACSTAFAYAGIDGISSNESNIKIGAAANASHPGGVAAVSVQAAGAPYNAFTGFSSLKGLAQAFAAQGTSNTNVTVGSKTFNISHIPVSAMPPSHSALGNFNFGQVGTQEVYFGEWWKAGDTPASASHTVYYAGDNTNTTVPTAGTATYTVAGINGSGSNLLSGTFTANYGAGTLEGTLTGTGTAVSSLSLDGVAFNPGTAAFAGLATANGTAGIDNSGVVQGQFFGANASALAGIAQFDNVSYNTAFGGAKN

SEQ ID NO: 20 - protein, 214 aa, Flavobacterium psychrophilum
MKNHFFKVAVLALTIFVSSCSKDEPATAVLTPQPQITTLEVKTVSNLNAPQVGMSFGPVSGEFTKFSFSENAVVTNDNWDVAFRGTTILVNGGAAIGIAGEPSRTGMGAVSIANNTLSGVTAFPAADTFRQDANSSYAIPIGSGNGWYNYNGATNIVTPLAGKVFVVKTHNGKYAKFEILSYYKDTPANPDAATSVGRHYTFKFVYQANSTTSF

SEQ ID NO: 21 - protein, 136 aa, Mycobacterium tuberculosis
MKTGTATTRRRLLAVLIALALPGAAVALLAEPSATGASDPCAASEVARTVGSVAKSMGDYLDSHPETNQVMTAVLQQQVGPGSVASLKAHFEANPKVASDLHALSQPLTDLSTRCSLPISGLQAIGLMQAVQGARR

SEQ ID NO: 22 - protein, 205 aa, Pseudomonas aeruginosa
MSISISYSTTYSGWTVADYLADWSAYFGDVNHRPGQVVDGANTGGFNPGPFDGSQYALKSTASDAAFIAGGDLHYTLFSNPSHTLWGKLDSIALGDTLTGGASSGGYTLDSQEVSFGNLGLDSPIAQGRDGTVHKVVYGLMSGDSSALQGQIDALLKAVDPSLSINSTFDQLAAAGVAHATPATAAADVGLVGVQELPQDLALAA

SEQ ID NO: 23 - protein, 189 aa, Alkalitalea saponilacus
MKTVLSLITLSWILVACSTSPGQDSQQSNSLSETEQQFLDNLKSLCGQSFEGRETYTKDGRDSWADKRMVIFFTVCESDEVHIPFHIDDDTSRTWMFINDHGSLRFRHDHRHPDGTPEDLTLYGGYSDGTGTPFRQSFPADQYTDNLLDDELDRVWNVILSDDLSTMTYELGYLGEIVFRAEFDLSNPL